European Patent Specification EP 3 137 506 B1, published August 30, 2023. Title: COMPOSITIONS AND METHODS RELATED TO ENGINEERED Fc CONSTRUCTS. Applicant: Momenta Pharmaceuticals, Inc. Bosques, Carlos J. Huston, James S. Lansing, Jonathan C. Ling, Leona E. Meador, James III Ortiz, Daniel Rutitzky, Laura Schultes, Brigit C. The sequence listing filed with the application follows.

SEQUENCE LISTING (46 sequences)

SEQ ID NO: 1 - protein, 5 aa, Artificial Sequence
  Synthetic Construct
GGGGS

SEQ ID NO: 2 - protein, 4 aa, Artificial Sequence
  Synthetic Construct
GGSG

SEQ ID NO: 3 - protein, 4 aa, Artificial Sequence
  Synthetic Construct
SGGG

SEQ ID NO: 4 - protein, 4 aa, Artificial Sequence
  Synthetic Construct
GSGS

SEQ ID NO: 5 - protein, 6 aa, Artificial Sequence
  Synthetic Construct
GSGSGS

SEQ ID NO: 6 - protein, 8 aa, Artificial Sequence
  Synthetic Construct
GSGSGSGS

SEQ ID NO: 7 - protein, 10 aa, Artificial Sequence
  Synthetic Construct
GSGSGSGSGS

SEQ ID NO: 8 - protein, 12 aa, Artificial Sequence
  Synthetic Construct
GSGSGSGSGSGS

SEQ ID NO: 9 - protein, 6 aa, Artificial Sequence
  Syntheic Construct
GGSGGS

SEQ ID NO: 10 - protein, 9 aa, Artificial Sequence
  Synthetic Construct
GGSGGSGGS

SEQ ID NO: 11 - protein, 12 aa, Artificial Sequence
  Synthetic Construct
GGSGGSGGSGGS

SEQ ID NO: 12 - protein, 4 aa, Artificial Sequence
  Synthetic Construct
GGSG

SEQ ID NO: 13 - protein, 4 aa, Artificial Sequence
  Synthetic Construct
GGSG

SEQ ID NO: 14 - protein, 8 aa, Artificial Sequence
  Synthetic Construct
GGSGGGSG

SEQ ID NO: 15 - protein, 12 aa, Artificial Sequence
  Synthetic Construct
GGSGGGSGGGSG

SEQ ID NO: 16 - protein, 5 aa, Artificial Sequence
  Synthetic Construct
GGGGS

SEQ ID NO: 17 - protein, 15 aa, Artificial Sequence
  Synthetic Construct
GGGGSGGGGSGGGGS

SEQ ID NO: 18 - protein, 10 aa, Artificial Sequence
  Synthetic Construct
GENLYFQSGG

SEQ ID NO: 19 - protein, 8 aa, Artificial Sequence
  Synthetic Construct
SACYCELS

SEQ ID NO: 20 - protein, 5 aa, Artificial Sequence
  Synthetic Construct
RSIAT

SEQ ID NO: 21 - protein, 17 aa, Artificial Sequence
  Synthetic Construct
RPACKIPNDLKQKVMNH

SEQ ID NO: 22 - protein, 36 aa, Artificial Sequence
  Synthetic Construct
GGSAGGSGSGSSGGSSGASGTGTAGGTGSGSGTGSG

SEQ ID NO: 23 - protein, 17 aa, Artificial Sequence
  Synthetic Construct
AAANSSIDLISVPVDSR

SEQ ID NO: 24 - protein, 36 aa, Artificial Sequence
  Synthetic Construct
GGSGGGSEGGGSEGGGSEGGGSEGGGSEGGGSGGGS

SEQ ID NO: 25 - protein, 12 aa, Artificial Sequence
  Synthetic Construct
GGGSGGGSGGGS

SEQ ID NO: 26 - protein, 20 aa, Artificial Sequence
  Synthetic Construct
SGGGSGGGSGGGSGGGSGGG

SEQ ID NO: 27 - protein, 18 aa, Artificial Sequence
  Synthetic Construct
GGSGGGSGGGSGGGSGGS

SEQ ID NO: 28 - protein, 11 aa, Artificial Sequence
  Synthetic Construct
DICLPRWGCLW

SEQ ID NO: 29 - DNA, 681 bp, Homo sapiens
gacaagacccacacctgtccgccttgccctgcccctgagctgctgggaggccccagcgtgttcctgttccccccaaagcccaaggacaccctgatgatcagccggacccccgaagtgacctgcgtggtggtggacgtgtcccacgaggaccctgaagtgaagttcaattggtacgtggacggcgtggaagtgcacaacgccaagaccaagcccagagaggaacagtacaacagcacctaccgggtggtgtccgtgctgaccgtgctgcaccaggactggctgaacggcaaagaatacaagtgcaaagtctccaacaaggccctgcctgcccccatcgagaaaaccatcagcaaggccaagggccagccccgcgagccccaggtgtacacactgccccccagccgggacgagctgaccaagaaccaggtgtccctgacctgcctggtgaaaggcttctaccccagcgatatcgccgtggaatgggagagcaacggccagcccgagaacaactacaagaccaccccccctgtgctggacagcgacggctcattcttcctgtacagcaagctgaccgtggacaagagccggtggcagcagggcaacgtgttcagctgcagcgtgatgcacgaggccctgcacaaccactacacccagaagtccctgagcctgagccccggcaag

SEQ ID NO: 30 - protein, 227 aa, Homo sapiens
DKTHTCPPCPAPELLGGPSVFLFPPKPKDTLMISRTPEVTCVVVDVSHEDPEVKFNWYVDGVEVHNAKTKPREEQYNSTYRVVSVLTVLHQDWLNGKEYKCKVSNKALPAPIEKTISKAKGQPREPQVYTLPPSRDELTKNQVSLTCLVKGFYPSDIAVEWESNGQPENNYKTTPPVLDSDGSFFLYSKLTVDKSRWQQGNVFSCSVMHEALHNHYTQKSLSLSPGK

SEQ ID NO: 31 - DNA, 681 bp, Artificial Sequence
  Synthetic Construct
gacaagacccacacctgtccgccttgccctgcccctgagctgctgggaggccccagcgtgttcctgttccccccaaagcccaaggacaccctgatgatcagccggacccccgaagtgacctgcgtggtggtggacgtgtcccacgaggaccctgaagtgaagttcaattggtacgtggacggcgtggaagtgcacaacgccaagaccaagcccagagaggaacagtacaacagcacctaccgggtggtgtccgtgctgaccgtgctgcaccaggactggctgaacggcaaagaatacaagtgcaaagtctccaacaaggccctgcctgcccccatcgagaaaaccatcagcaaggccaagggccagccccgcgagccccaggtgtacacactgcccccctgccgggacgagctgaccaagaaccaggtgtccctgtggtgcctggtgaaaggcttctaccccagcgatatcgccgtggaatgggagagcaacggccagcccgagaacaactacaagaccaccccccctgtgctggacagcgacggctcattcttcctgtacagcaagctgaccgtggacaagagccggtggcagcagggcaacgtgttcagctgcagcgtgatgcacgaggccctgcacaaccactacacccagaagtccctgagcctgagccccggcaag

SEQ ID NO: 32 - protein, 227 aa, Artificial Sequence
  Synthetic Construct
DKTHTCPPCPAPELLGGPSVFLFPPKPKDTLMISRTPEVTCVVVDVSHEDPEVKFNWYVDGVEVHNAKTKPREEQYNSTYRVVSVLTVLHQDWLNGKEYKCKVSNKALPAPIEKTISKAKGQPREPQVYTLPPCRDELTKNQVSLWCLVKGFYPSDIAVEWESNGQPENNYKTTPPVLDSDGSFFLYSKLTVDKSRWQQGNVFSCSVMHEALHNHYTQKSLSLSPGK

SEQ ID NO: 33 - DNA, 681 bp, Artificial Sequence
  Synthetic Construct
gacaagacccacacctgtccgccttgccctgcccctgagctgctgggaggccccagcgtgttcctgttccccccaaagcccaaggacaccctgatgatcagccggacccccgaagtgacctgcgtggtggtggacgtgtcccacgaggaccctgaagtgaagttcaattggtacgtggacggcgtggaagtgcacaacgccaagaccaagcccagagaggaacagtacaacagcacctaccgggtggtgtccgtgctgaccgtgctgcaccaggactggctgaacggcaaagaatacaagtgcaaagtctccaacaaggccctgcctgcccccatcgagaaaaccatcagcaaggccaagggccagccccgcgagccccaagtgtgtacactgccccccagccgggacgagctgaccaagaaccaggtgtccctgagctgcgccgtgaaaggcttctaccccagcgatatcgccgtggaatgggagagcaacggccagcccgagaacaactacaagaccaccccccctgtgctggacagcgacggctcattcttcctggttagcaagctgaccgtggacaagagccggtggcagcagggcaacgtgttcagctgcagcgtgatgcacgaggccctgcacaaccactacacccagaagtccctgagcctgagccccggcaag

SEQ ID NO: 34 - protein, 227 aa, Artificial Sequence
  Synthetic Construct
DKTHTCPPCPAPELLGGPSVFLFPPKPKDTLMISRTPEVTCVVVDVSHEDPEVKFNWYVDGVEVHNAKTKPREEQYNSTYRVVSVLTVLHQDWLNGKEYKCKVSNKALPAPIEKTISKAKGQPREPQVCTLPPSRDELTKNQVSLSCAVKGFYPSDIAVEWESNGQPENNYKTTPPVLDSDGSFFLVSKLTVDKSRWQQGNVFSCSVMHEALHNHYTQKSLSLSPGK

SEQ ID NO: 35 - DNA, 681 bp, Artificial Sequence
  Synthetic Construct
gacaagacccacacctgtccgccttgccctgcccctgagctgctgggaggccccagcgtgttcctgttccccccaaagcccaaggacaccctgatgatcagccggacccccgaagtgacctgcgtggtggtggacgtgtcccacgaggaccctgaagtgaagttcaattggtacgtggacggcgtggaagtgcacaacgccaagaccaagcccagagaggaacagtacaacagcacctaccgggtggtgtccgtgctgaccgtgctgcaccaggactggctgaacggcaaagaatacaagtgcaaagtctccaacaaggccctgcctgcccccatcgagaaaaccatcagcaaggccaagggccagccccgcgagccccaggtgtacacactgccccccagccgggacgagctgaccaagaaccaggtgtccctgacctgcctggtgaaaggcttctaccccagcgatatcgccgtggaatgggagagcaacggccagcccgagaacaactacaagaccaccccccctgtgctgaaaagcgacggctcattcttcctgtacagcgacctgaccgtggacaagagccggtggcagcagggcaacgtgttcagctgcagcgtgatgcacgaggccctgcacaaccactacacccagaagtccctgagcctgagccccggcaag

SEQ ID NO: 36 - protein, 227 aa, Artificial Sequence
  Synthetic Construct
DKTHTCPPCPAPELLGGPSVFLFPPKPKDTLMISRTPEVTCVVVDVSHEDPEVKFNWYVDGVEVHNAKTKPREEQYNSTYRVVSVLTVLHQDWLNGKEYKCKVSNKALPAPIEKTISKAKGQPREPQVYTLPPSRDELTKNQVSLTCLVKGFYPSDIAVEWESNGQPENNYKTTPPVLKSDGSFFLYSDLTVDKSRWQQGNVFSCSVMHEALHNHYTQKSLSLSPGK

SEQ ID NO: 37 - DNA, 1398 bp, Artificial Sequence
  Synthetic Construct
gacaagacccacacctgtcccccttgccctgcccctgagctgctgggaggccccagcgtgttcctgttccccccaaagcccaaggacaccctgatgatcagccggacccccgaagtgacctgcgtggtggtggacgtgtcccacgaggaccctgaagtgaagttcaattggtacgtggacggcgtggaagtgcacaacgccaagaccaagcccagagaggaacagtacaacagcacctaccgggtggtgtccgtgctgaccgtgctgcaccaggactggctcaacggcaaagagtacaagtgcaaggtgtccaacaaggccctgcctgcccccatcgagaaaaccatcagcaaggccaagggccagccccgcgagccccaggtctacacactgccccccagccgggacgagctgaccaagaaccaggtctccctgacctgcctggtgaaaggcttctaccccagcgatatcgccgtggaatgggagagcaacggccagcccgagaacaactacaagaccaccccccctgtgctggacagcgacggctcattcttcctgtacagcaagctgaccgtggacaagagccggtggcagcagggcaacgtgttcagctgcagcgtgatgcacgaggccctgcacaaccactacacccagaagtccctgagcctgagccccggcaaaggcgggggatctgggggaggaagcggaggcggcagcgataagacccatacctgccctccctgtcccgctcccgaactgctggggggaccctccgtgtttctgtttccacctaagcctaaggatacgctcatgatctccagaacccctgaagtcacatgtgtggtggtcgatgtgtctcatgaagatcccgaagtcaagtttaactggtatgtggatggggtcgaggtccacaatgccaaaacaaagcctcgggaagaacagtataactccacctacagagtcgtcagcgtgctgacagtccttcatcaggattggctgaatgggaaagagtacaaatgtaaagtgtctaacaaagctctgcccgctcctatcgaaaagaccatctccaaagccaaagggcagcccagagaacctcaggtgtacaccctgccaccctccagagatgagctgacaaaaaatcaggtgtcactgacatgtctggtgaaagggttttatccctccgacattgctgtggaatgggaatccaatgggcagcctgaaaacaattataagacaacacctcccgtgctggactccgatggctcattttttctgtactctaaactgacagtggataagtccagatggcagcagggaaatgtgttttcctgctctgtgatgcatgaagctctgcataatcactatacacagaaaagcctgtccctgtcccccggcaag

SEQ ID NO: 38 - protein, 466 aa, Artificial Sequence
  Synthetic Construct
DKTHTCPPCPAPELLGGPSVFLFPPKPKDTLMISRTPEVTCVVVDVSHEDPEVKFNWYVDGVEVHNAKTKPREEQYNSTYRVVSVLTVLHQDWLNGKEYKCKVSNKALPAPIEKTISKAKGQPREPQVYTLPPSRDELTKNQVSLTCLVKGFYPSDIAVEWESNGQPENNYKTTPPVLDSDGSFFLYSKLTVDKSRWQQGNVFSCSVMHEALHNHYTQKSLSLSPGKGGGSGGGSGGGSDKTHTCPPCPAPELLGGPSVFLFPPKPKDTLMISRTPEVTCVVVDVSHEDPEVKFNWYVDGVEVHNAKTKPREEQYNSTYRVVSVLTVLHQDWLNGKEYKCKVSNKALPAPIEKTISKAKGQPREPQVYTLPPSRDELTKNQVSLTCLVKGFYPSDIAVEWESNGQPENNYKTTPPVLDSDGSFFLYSKLTVDKSRWQQGNVFSCSVMHEALHNHYTQKSLSLSPGK

SEQ ID NO: 39 - DNA, 1422 bp, Artificial Sequence
  Synthetic Construct
gacaagacccacacctgtcccccttgcccagcccctgagctgctgggaggccccagcgtgttcctgttccccccaaagcccaaggacaccctgatgatcagccggacccccgaagtgacctgcgtggtggtggacgtgtcccacgaggaccctgaagtgaagttcaattggtacgtggacggcgtggaagtgcacaacgccaagaccaagcccagagaggaacagtacaacagcacctaccgggtggtgtccgtgctgaccgtgctgcaccaggactggctgaacggcaaagagtacaagtgcaaggtgtccaacaaggccctgcctgcccccatcgagaaaaccatcagcaaggccaagggccagccccgcgagccccaggtgtacaccctgcccccttgcagagatgagctgaccaagaaccaggtgtccctgtggtgcctggtcaagggcttctaccccagcgatatcgccgtggaatgggagagcaacggccagcccgagaacaactacaagaccaccccccctgtgctggacagcgacggctcattcttcctgtacagcaagctgaccgtggacaagagccggtggcagcagggcaacgtgttcagctgcagcgtgatgcacgaggccctgcacaaccactacacccagaagtccctgagcctgagccccggcaagtctgggggaggatcagggggtggaagtggcggtggatctggtggtggaagcggaggcggcgataagacacacacatgccccccctgtccagctcccgaactgctggggggaccctccgtgtttctgtttccacctaagcctaaggatacgctcatgatctccagaacccctgaagtcacatgtgtggtggtcgatgtgtctcatgaagatcccgaagtcaagtttaattggtatgtcgatggggtcgaggtgcacaatgccaaaacaaaacctcgggaagaacagtataactccacatacagagtggtgtctgtcctcacagtcctgcatcaggattggctcaatgggaaagagtacaaatgtaaagtctctaacaaggctctccccgctccgatcgaaaagaccatctccaaagccaaagggcagcccagagaacctcaggtctacacactgcctcccagccgggacgagctgacaaaaaatcaagtgtctctgacctgcctcgtgaagggcttttatccctccgacattgccgtcgagtgggagtccaatggacagccggaaaacaattataagaccacgcctccagtgctgaagtccgacggcagcttctttctgtactccgacctgacagtggataagtccagatggcagcaagggaatgtgttctcctgttccgtgatgcatgaagccctccataatcactatacccagaaaagcctgtccctgtcccctggcaag

SEQ ID NO: 40 - protein, 474 aa, Artificial Sequence
  Synthetic Construct
DKTHTCPPCPAPELLGGPSVFLFPPKPKDTLMISRTPEVTCVVVDVSHEDPEVKFNWYVDGVEVHNAKTKPREEQYNSTYRVVSVLTVLHQDWLNGKEYKCKVSNKALPAPIEKTISKAKGQPREPQVYTLPPCRDELTKNQVSLWCLVKGFYPSDIAVEWESNGQPENNYKTTPPVLDSDGSFFLYSKLTVDKSRWQQGNVFSCSVMHEALHNHYTQKSLSLSPGKSGGGSGGGSGGGSGGGSGGGDKTHTCPPCPAPELLGGPSVFLFPPKPKDTLMISRTPEVTCVVVDVSHEDPEVKFNWYVDGVEVHNAKTKPREEQYNSTYRVVSVLTVLHQDWLNGKEYKCKVSNKALPAPIEKTISKAKGQPREPQVYTLPPSRDELTKNQVSLTCLVKGFYPSDIAVEWESNGQPENNYKTTPPVLKSDGSFFLYSDLTVDKSRWQQGNVFSCSVMHEALHNHYTQKSLSLSPGK

SEQ ID NO: 41 - DNA, 1422 bp, Artificial Sequence
  Synthetic Construct
gacaagacccacacctgtcccccttgccctgcccctgagctgctgggaggccccagcgtgttcctgttccccccaaagcccaaggacaccctgatgatcagccggacccccgaagtgacctgcgtggtggtggacgtgtcccacgaggaccctgaagtgaagttcaattggtacgtggacggcgtggaagtgcacaacgccaagaccaagcccagagaggaacagtacaacagcacctaccgggtggtgtccgtgctgaccgtgctgcaccaggactggctgaacggcaaagagtacaagtgcaaggtgtccaacaaggccctgcctgcccccatcgagaaaaccatcagcaaggccaagggccagccccgcgagccccaggtgtacaccctgcccccttgcagagatgaactgaccaagaaccaggtgtccctgtggtgcctggtcaagggcttctaccccagcgatatcgccgtggaatgggagagcaacggccagcccgagaacaactacaagaccaccccccctgtgctggacagcgacggctcattcttcctgtacagcaagctgaccgtggacaagagccggtggcagcagggcaacgtgttcagctgcagcgtgatgcacgaggccctgcacaaccactacacccagaagtccctgagcctgagccccggcaagtctgggggaggatcagggggtggaagtggcggtggatctggtggtggaagcggaggcggcgataagacacacacatgccccccctgtccagctcccgaactgctggggggaccctccgtgtttctgtttccacctaagcctaaggatacgctcatgatctccagaacccctgaagtcacatgtgtggtggtcgatgtgtctcatgaagatcccgaagtcaagtttaactggtatgtggatggggtcgaggtccacaatgccaaaacaaagcctcgggaagaacagtataactccacctacagagtcgtcagcgtgctgacagtcctgcatcaagattggctcaatgggaaagagtataagtgtaaagtctcgaacaaagccctccccgctcctatcgaaaagaccatctccaaagccaaagggcagcccagagaacctcaggtctacacactgcctccatgtcgggacgagctgacaaaaaatcaggtgtcactgtggtgtctggtgaaggggttttacccttccgacattgctgtggaatgggaatccaatgggcagcctgaaaacaattataagacaacacctcccgtgctggactccgatggctcattttttctgtactctaaactgacagtggataagtccagatggcagcagggaaatgtgttttcctgctctgtgatgcatgaagctctgcataatcactatacacagaaaagcctgtccctgtcccctggcaag

SEQ ID NO: 42 - protein, 474 aa, Artificial Sequence
  Synthetic Construct
DKTHTCPPCPAPELLGGPSVFLFPPKPKDTLMISRTPEVTCVVVDVSHEDPEVKFNWYVDGVEVHNAKTKPREEQYNSTYRVVSVLTVLHQDWLNGKEYKCKVSNKALPAPIEKTISKAKGQPREPQVYTLPPCRDELTKNQVSLWCLVKGFYPSDIAVEWESNGQPENNYKTTPPVLDSDGSFFLYSKLTVDKSRWQQGNVFSCSVMHEALHNHYTQKSLSLSPGKSGGGSGGGSGGGSGGGSGGGDKTHTCPPCPAPELLGGPSVFLFPPKPKDTLMISRTPEVTCVVVDVSHEDPEVKFNWYVDGVEVHNAKTKPREEQYNSTYRVVSVLTVLHQDWLNGKEYKCKVSNKALPAPIEKTISKAKGQPREPQVYTLPPCRDELTKNQVSLWCLVKGFYPSDIAVEWESNGQPENNYKTTPPVLDSDGSFFLYSKLTVDKSRWQQGNVFSCSVMHEALHNHYTQKSLSLSPGK

SEQ ID NO: 43 - DNA, 1365 bp, Artificial Sequence
  Synthetic Construct
aggacagtggccgctcccagcgtgttcatcttcccacccagcgacgagcagctgaagtccggcacagccagcgtggtctgcctgctgaacaacttctacccccgcgaggccaaggtgcagtggaaggtggacaacgccctgcagagcggcaacagccaggaaagcgtcaccgagcaggacagcaaggactccacctacagcctgtctagcaccctgaccctgagcaaggccgactacgagaagcacaaggtgtacgcctgcgaagtgacccaccagggcctgtccagccccgtgaccaagagcttcaacagaggcgagtgcggcggctctggcggaggatccgggggaggatcaggcggcggaagcggaggcagcgctagcacaaagggcccctccgtgttccccctggcccccagcagcaagagcacatctggcggaacagccgccctgggctgcctggtgaaagactacttccccgagcccgtgaccgtgtcctggaactctggcgccctgaccagcggcgtgcacacctttccagccgtgctgcagagcagcggcctgtactccctgagcagcgtggtgacagtgcctagcagcagcctgggcacccagacctacatctgcaacgtgaaccacaagcccagcaacaccaaagtggacaagcgggtggaacccaagagctgcgacaagacccacacgtgtcccccctgcccagcccctgaactgctgggcggacctagcgtgttcctgttccccccaaagcccaaggacaccctgatgatcagccggacccccgaagtgacctgcgtggtggtggacgtgtcccacgaggaccctgaagtgaagttcaattggtacgtggacggcgtggaagtgcacaatgccaagaccaagcccagagaggaacagtacaacagcacctaccgggtggtgtccgtgctgaccgtgctgcaccaggactggctgaacggcaaagagtacaagtgcaaggtctccaacaaggccctgcctgcccccatcgagaaaaccatcagcaaggccaagggccagccccgcgagccccaggtgtacacactgccccccagccgggacgagctgaccaagaaccaggtgtccctgacctgtctggtgaaaggcttctacccctccgatatcgccgtggaatgggagagcaacggccagcccgagaacaactacaagaccaccccccctgtgctggactccgacggctcattcttcctgtacagcaagctgaccgtggacaagagccggtggcagcagggcaacgtgttcagctgctccgtgatgcacgaggccctgcacaaccactacacccagaagtccctgagcctgagccccggcaaa

SEQ ID NO: 44 - protein, 455 aa, Artificial Sequence
  Synthetic Construct
RTVAAPSVFIFPPSDEQLKSGTASVVCLLNNFYPREAKVQWKVDNALQSGNSQESVTEQDSKDSTYSLSSTLTLSKADYEKHKVYACEVTHQGLSSPVTKSFNRGECGGSGGGSGGGSGGGSGGSASTKGPSVFPLAPSSKSTSGGTAALGCLVKDYFPEPVTVSWNSGALTSGVHTFPAVLQSSGLYSLSSVVTVPSSSLGTQTYICNVNHKPSNTKVDKRVEPKSCDKTHTCPPCPAPELLGGPSVFLFPPKPKDTLMISRTPEVTCVVVDVSHEDPEVKFNWYVDGVEVHNAKTKPREEQYNSTYRVVSVLTVLHQDWLNGKEYKCKVSNKALPAPIEKTISKAKGQPREPQVYTLPPSRDELTKNQVSLTCLVKGFYPSDIAVEWESNGQPENNYKTTPPVLDSDGSFFLYSKLTVDKSRWQQGNVFSCSVMHEALHNHYTQKSLSLSPGK

SEQ ID NO: 45 - protein, 227 aa, Artificial Sequence
  Synthetic Construct
DKTHTCPPCPAPELLGGPSVFLFPPKPKDTLMISRTPEVTCVVVDVSHEDPEVKFNWYVDGVEVHNAKTKPREEQYNSTYRVVSVLTVLHQDWLNGKEYKCKVSNKALPAPIEKTISKAKGQPREPQVCTLPPSRDELTKNQVSLSCAVEGFYPSDIAVEWESNGQPENNYKTTPPVLDSDGSFFLVSKLTVDKSRWQQGNVFSCSVMHEALHNHYTQKSLSLSPGK

SEQ ID NO: 46 - protein, 474 aa, Artificial Sequence
  Synthetic Construct
DKTHTCPPCPAPELLGGPSVFLFPPKPKDTLMISRTPEVTCVVVDVSHEDPEVKFNWYVDGVEVHNAKTKPREEQYNSTYRVVSVLTVLHQDWLNGKEYKCKVSNKALPAPIEKTISKAKGQPREPQVYTLPPCRDKLTKNQVSLWCLVKGFYPSDIAVEWESNGQPENNYKTTPPVLDSDGSFFLYSKLTVDKSRWQQGNVFSCSVMHEALHNHYTQKSLSLSPGKSGGGSGGGSGGGSGGGSGGGDKTHTCPPCPAPELLGGPSVFLFPPKPKDTLMISRTPEVTCVVVDVSHEDPEVKFNWYVDGVEVHNAKTKPREEQYNSTYRVVSVLTVLHQDWLNGKEYKCKVSNKALPAPIEKTISKAKGQPREPQVYTLPPSRDELTKNQVSLTCLVKGFYPSDIAVEWESNGQPENNYKTTPPVLKSDGSFFLYSDLTVDKSRWQQGNVFSCSVMHEALHNHYTQKSLSLSPGK